European Patent Specification EP 4 204 570 B1, published June 4, 2025. Title: METHOD OF PRODUCING A RECOMBINANT PROTEIN IN A HOST CELL WHICH HAS A DISABLED RHAMNOSE METABOLISM AS WELL AS EXPRESSION VECTORS, HOST CELLS AND RECOMBINANT PROTEINS THEREOF. Applicant: Xbrane Biopharma AB STADA Arzneimittel AG. The sequence listing filed with the application follows.

SEQUENCE LISTING (21 sequences)

SEQ ID NO: 1 - DNA, 4673 bp, Artificial Sequence
  KTXHIS
atctttctgcgaattgagatgacgccactggctgggcgtcatcccggtttcccgggtaaacaccaccgaaaaatagttactatcttcaaagccacattcggtcgaaatatcactgattaacaggcggctatgctggagaagatattgcgcatgacacactctgacctgtcgcagatattgattgatggtcattccagtctgctggcgaaattgctgacgcaaaacgcgctcactgcacgatgcctcatcacaaaatttatccagcgcaaagggacttttcaggctagccgccagccgggtaatcagcttatccagcaacgtttcgctggatgttggcggcaacgaatcactggtgtaacgatggcgattcagcaacatcaccaactgcccgaacagcaactcagccatttcgttagcaaacggcacatgctgactactttcatgctcaagctgaccaataacctgccgcgcctgcgccatccccatgctacctaagcgccagtgtggttgccctgcgctggcgttaaatcccggaatcgccccctgccagtcaagattcagcttcagacgctccgggcaataaataatattctgcaaaaccagatcgttaacggaagcgtaggagtgtttatcatcagcatgaatgtaaaagagatcgccacgggtaatgcgataagggcgatcgttgagtacatgcaggccattaccgcgccagacaatcaccagctcacaaaaatcatgtgtatgttcagcaaagacatcttgcggataacggtcagccacagcgactgcctgctggtcgctggcaaaaaaatcatctttgagaagttttaactgatgcgccaccgtggctacctcggccagagaacgaagttgattattcgcaatatggcgtacaaatacgttgagaagattcgcgttattgcagaaagccatcccgtccctggcgaatatcacgcggtgaccagttaaactctcggcgaaaaagcgtcgaaaagtggttactgtcgctgaatccacagcgataggcgatgtcagtaacgctggcctcgctgtggcgtagcagatgtcgggctttcatcagtcgcaggcggttcaggtatcgctgaggcgtcagtcccgtttgctgcttaagctgccgatgtagcgtacgcagtgaaagagaaaattgatccgccacggcatcccaattcacctcatcggcaaaatggtcctccagccaggccagaagcaagttgagacgtgatgcgctgttttccaggttctcctgcaaactgcttttacgcagcaagagcagtaattgcataaacaagatctcgcgactggcggtcgagggtaaatcattttccccttcctgctgttccatctgtgcaaccagctgtcgcacctgctgcaatacgctgtggttaacgcgccagtgagacggatactgcccatccagctcttgtggcagcaactgattcagcccggcgagaaactgaaatcgatccggcgagcgatacagcacattggtcagacacagattatcggtatgttcatacagatgccgatcatgatcgcgtacgaaacagaccgtgccaccggtgatggtatagggctgcccattaaacacatgaatacccgtgccatgttcgacaatcacaatttcatgaaaatcatgatgatgttcaggaaaatccgcctgcgggagccggggttctatcgccacggacgcgttaccagacggaaaaaaatccacactatgtaatacggtcatactggcctcctgatgtcgtcaacacggcgaaatagtaatcacgaggtcaggttcttaccttaaattttcgacggaaaaccacgtaaaaaacgtcgatttttcaagatacagcgtgaattttcaggaaatgcggtgagcatcacatcaccacaattcagcaaattgtgaacatcatcacgttcatctttccctggttgccaatggcccattttcttgtcagtaacgagaaggtcgcgaatccaggcgctttttagactggtcgtaatgaaattcaggaggaattccatatggcggccgcactcgagcaccaccaccaccaccactgatgaagacggccgcctaggggtaccgagctcggatcctctagagtcgacctgcaggcatgcaagcttggctgttttggcggatgagagaagattttcagcctgatacagattaaatcagaacgcagaagcggtctgataaaacagaatttgcctggcggcagtagcgcggtggtcccacctgaccccatgccgaactcagaagtgaaacgccgtagcgccgatggtagtgtggggtctccccatgcgagagtagggaactgccaggcatcaaataaaacgaaaggctcagtcgaaagactgggcctttcgttttatctgttgtttgtcggtgaacgctctcctgagtaggacaaatccgccgggagcggatttgaacgttgcgaagcaacggcccggagggtggcgggcaggacgcccgccataaactgccaggcatcaaattaagcagaaggccatcctgacggatggcctttttgcgtttctacaaactcttttgtttatttttctaaatacattcaaatatgtatccgctcatgagactaggcttccgcgccctcatccgaaagggcgtattcatatatgcggtgtgaaataccgcacagatgcgtaaggagaaaataccgcatcaggcgctcttccgcttcctcgctcactgactcgctgcgctcggtcgttcggctgcggcgagcggtatcagctcactcaaaggcggtaatacggttatccacagaatcaggggataacgcaggaaagaacatgtgagcaaaaggccagcaaaaggccaggaaccgtaaaaaggccgcgttgctggcgtttttccataggctccgcccccctgacgagcatcacaaaaatcgacgctcaagtcagaggtggcgaaacccgacaggactataaagataccaggcgtttccccctggaagctccctcgtgcgctctcctgttccgaccctgccgcttaccggatacctgtccgcctttctcccttcgggaagcgtggcgctttctcatagctcacgctgtaggtatctcagttcggtgtaggtcgttcgctccaagctgggctgtgtgcacgaaccccccgttcagcccgaccgctgcgccttatccggtaactatcgtcttgagtccaacccggtaagacacgacttatcgccactggcagcagccactggtaacaggattagcagagcgaggtatgtaggcggtgctacagagttcttgaagtggtggcctaactacggctacactagaaggacagtatttggtatctgcgctctgctgaagccagttaccttcggaaaaagagttggtagctcttgatccggcaaacaaaccaccgctggtagcggtggtttttttgtttgcaagcagcagattacgcgcagaaaaaaaggatctcaagaagatcctttgatcttttctacggggtctgacgctcagtggaacgaaaactcacgttaagggattttggtcatgagattatcaaaaaggatcttcacctagatccttttaaattaaaaatgaagttttaaatcaatctaaagtatatatgagtaaacttggtctgacagttagaaaaactcatcgagcatcaaatgaaactgcaatttattcatatcaggattatcaataccatatttttgaaaaagccgtttctgtaatgaaggagaaaactcaccgaggcagttccataggatggcaagatcctggtatcggtctgcgattccgactcgtccaacatcaatacaacctattaatttcccctcgtcaaaaataaggttatcaagtgagaaatcaccatgagtgacgactgaatccggtgagaatggcaaaagtttatgcatttctttccagacttgttcaacaggccagccattacgctcgtcatcaaaatcactcgcatcaaccaaaccgttattcattcgtgattgcgcctgagcgagacgaaatacgcgatcgctgttaaaaggacaattacaaacaggaatcgaatgcaaccggcgcaggaacactgccagcgcatcaacaatattttcacctgaatcaggatattcttctaatacctggaatgctgttttcccggggatcgcagtggtgagtaaccatgcatcatcaggagtacggataaaatgcttgatggtcggaagaggcataaattccgtcagccagtttagtctgaccatctcatctgtaacatcattggcaacgctacctttgccatgtttcagaaacaactctggcgcatcgggcttcccatacaatcgatagattgtcgcacctgattgcccgacattatcgcgagcccatttatacccatataaatcagcatccatgttggaatttaatcgcggcctagagcaagacgtttcccgttgaatatggctcatactcttcctttttcaatattattgaagcatttatcagggttattgtctcatgagcggatacatatttgaatgtatttagaaaaataaacaaataggggttccgcgcacatttccccgaaaagtgccacctgacgtctaagaaaccattattatcatgacattaacctataaaaataggcgtatcacgaggccctttcgtct

SEQ ID NO: 2 - DNA, 767 bp, Artificial Sequence
  frame shift mutation
gttggccccgctccacgccagtagcgactcgtcccagtcgtcgctattgatattgaccagttgcgtggtcgtggcgttggtatattcccagttcatcttgccggtcaggcgataactgaagtaatccggcatcagcagagcgtgagcaatgtgtggaataagttcaggttgttgctccgtcagcgcacgcaactgataaagcgtattgaagggcagaaactggatgccgctacgttgataaatatcgcgtttgccgagttgttgttgtgcctgcgccattaggccattggtgcggctatcgcgataagcaacgggcaggcccacacgctgaccctgttggtcgagcagcacaaagtccacgccccaggtatcaatcccaatgctatcgcgatacgaatcccttcctcgcacaccttgtttaatccaaggcgaatggcactttccaggctatccacatcccaggtgacatagccgttctgactatgcagcccattgttaaaacgatggatttcgcgcagcgtcaggctgcggcattcacgctcgtaacgcgccagcatcacgcgcccactggatgcgccgagatcgacggcgacacaattgcgaaaggtcataatgtgatcctgctgaatttcattacgaccagtctaaaaagcgcctgaattcgcgaccttctcgttactgacaggaaaatgggccattggcaaccagggaaagatgaacgtgatgatgttcacaatttgctgaattgtggtgatgtgatgctcacc

SEQ ID NO: 3 - protein, 214 aa, Artificial Sequence
  Ranibizumab light chain
DIQLTQSPSSLSASVGDRVTITCSASQDISNYLNWYQQKPGKAPKVLIYFTSSLHSGVPSRFSGSGSGTDFTLTISSLQPEDFATYYCQQYSTVPWTFGQGTKVEIKRTVAAPSVFIFPPSDEQLKSGTASVVCLLNNFYPREAKVQWKVDNALQSGNSQESVTEQDSKDSTYSLSSTLTLSKADYEKHKVYACEVTHQGLSSPVTKSFNRGEC

SEQ ID NO: 4 - protein, 231 aa, Artificial Sequence
  Ranibizumab heavy chain
EVQLVESGGGLVQPGGSLRLSCAASGYDFTHYGMNWVRQAPGKGLEWVGWINTYTGEPTYAADFKRRFTFSLDTSKSTAYLQMNSLRAEDTAVYYCAKYPYYYGTSHWYFDVWGQGTLVTVSSASTKGPSVFPLAPSSKSTSGGTAALGCLVKDYFPEPVTVSWNSGALTSGVHTFPAVLQSSGLYSLSSVVTVPSSSLGTQTYICNVNHKPSNTKVDKKVEPKSCDKTHL

SEQ ID NO: 5 - DNA, 645 bp, Artificial Sequence
  ranibizumab light chain
gatattcagctgacccagagcccgagcagcctgagcgcaagcgttggtgatcgtgttaccattacctgtagcgcaagccaggatattagcaattatctgaattggtatcagcagaaaccgggtaaagcaccgaaagtgctgatctattttaccagcagcctgcatagcggtgttccgagccgttttagcggtagcggtagtggcaccgattttaccctgaccattagcagcctgcagccggaagattttgcaacctattattgtcagcagtatagcaccgttccgtggacctttggtcagggcaccaaagttgaaattaaacgtaccgttgcagcaccgagcgtttttatctttccgcctagtgatgaacagctgaaaagcggcaccgcaagcgttgtttgtctgctgaataacttttatccgcgtgaagcaaaagttcagtggaaagttgataatgcactgcagagcggtaatagccaagaaagcgttaccgaacaggatagcaaagatagcacctatagcctgagcagcaccctgaccctgagcaaagcagattatgaaaaacacaaagtgtatgcctgcgaagttacccatcagggtctgagcagtccggttaccaaaagttttaatcgtggtgaatgctaa

SEQ ID NO: 6 - DNA, 696 bp, Artificial Sequence
  ranibizumab heavy chain
gaagttcagctggttgaaagcggtggtggtctggttcagcctggtggtagcctgcgtctgagctgtgcagcaagcggttatgattttacccattatggtatgaattgggttcgtcaggcaccgggtaaaggtctggaatgggttggttggattaatacctataccggtgaaccgacctatgcagcagattttaaacgtcgttttacctttagcctggataccagcaaaagcaccgcatatctgcagatgaatagcctgcgtgcagaggataccgcagtgtattattgtgcaaaatatccgtattattacggcaccagccattggtatttcgatgtttggggtcagggcaccctggttaccgttagcagcgcaagcaccaaaggtccgagcgtttttccgctggcaccgagcagcaaaagtaccagcggtggcaccgcagcactgggttgtctggttaaagattattttccggaaccggttaccgtgagctggaatagcggtgcactgaccagcggtgttcatacctttccggcagttctgcagagcagcggtctgtatagcctgagcagcgttgttaccgttccgagcagcagcctgggcacccagacctatatttgtaatgttaatcataaaccgagcaataccaaagtggataaaaaagtggaaccgaaaagctgcgataaaacccatctgtaa

SEQ ID NO: 7 - DNA, 66 bp, Artificial Sequence
  PelB signal peptide - DNA
atgaaatatctgctgccgaccgcagcagcgggtctgctgctgctggcagcacagcctgcaatggca

SEQ ID NO: 8 - DNA, 119 bp, Artificial Sequence
  rhaBAD promoter
caccacaattcagcaaattgtgaacatcatcacgttcatctttccctggttgccaatggcccattttcttgtcagtaacgagaaggtcgcgaatccaggcgctttttagactggtcgta

SEQ ID NO: 9 - DNA, 936 bp, Artificial Sequence
  RhaR transcription activator
atggctttctgcaataacgcgaatcttctcaacgtatttgtacgccatattgcgaataatcaacttcgttctctggccgaggtagccacggtggcgcatcagttaaaacttctcaaagatgatttttttgccagcgaccagcaggcagtcgctgtggctgaccgttatccgcaagatgtctttgctgaacatacacatgatttttgtgagctggtgattgtctggcgcggtaatggcctgcatgtactcaacgatcgcccttatcgcattacccgtggcgatctcttttacattcatgctgatgataaacactcctacgcttccgttaacgatctggttttgcagaatattatttattgcccggagcgtctgaagctgaatcttgactggcagggggcgattccgggatttaacgccagcgcagggcaaccacactggcgcttaggtagcatggggatggcgcaggcgcggcaggttattggtcagcttgagcatgaaagtagtcagcatgtgccgtttgctaacgaaatggctgagttgctgttcgggcagttggtgatgttgctgaatcgccatcgttacaccagtgattcgttgccgccaacatccagcgaaacgttgctggataagctgattacccggctggcggctagcctgaaaagtccctttgcgctggataaattttgtgatgaggcatcgtgcagtgagcgcgttttgcgtcagcaatttcgccagcagactggaatgaccatcaatcaatatctgcgacaggtcagagtgtgtcatgcgcaatatcttctccagcatagccgcctgttaatcagtgatatttcgaccgaatgtggctttgaagatagtaactatttttcggtggtgtttacccgggaaaccgggatgacgcccagccagtggcgtcatctcaattcgcagaaagat

SEQ ID NO: 10 - DNA, 36 bp, Artificial Sequence
  RhaR extended
agacgaaagggcctcgtgatacgcctatttttatag

SEQ ID NO: 11 - DNA, 837 bp, Artificial Sequence
  RhaS transcription activator
atgaccgtattacatagtgtggatttttttccgtctggtaacgcgtccgtggcgatagaaccccggctcccgcaggcggattttcctgaacatcatcatgattttcatgaaattgtgattgtcgaacatggcacgggtattcatgtgtttaatgggcagccctataccatcaccggtggcacggtctgtttcgtacgcgatcatgatcggcatctgtatgaacataccgataatctgtgtctgaccaatgtgctgtatcgctcgccggatcgatttcagtttctcgccgggctgaatcagttgctgccacaagagctggatgggcagtatccgtctcactggcgcgttaaccacagcgtattgcagcaggtgcgacagctggttgcacagatggaacagcaggaaggggaaaatgatttaccctcgaccgccagtcgcgagatcttgtttatgcaattactgctcttgctgcgtaaaagcagtttgcaggagaacctggaaaacagcgcatcacgtctcaacttgcttctggcctggctggaggaccattttgccgatgaggtgaattgggatgccgtggcggatcaattttctctttcactgcgtacgctacatcggcagcttaagcagcaaacgggactgacgcctcagcgatacctgaaccgcctgcgactgatgaaagcccgacatctgctacgccacagcgaggccagcgttactgacatcgcctatcgctgtggattcagcgacagtaaccacttttcgacgctttttcgccgagagtttaactggtcaccgcgtgatattcgccagggacgggatggctttctgcaataa

SEQ ID NO: 12 - DNA, 816 bp, Artificial Sequence
  KanR
atgagccatattcaacgggaaacgtcttgctctaggccgcgattaaattccaacatggatgctgatttatatgggtataaatgggctcgcgataatgtcgggcaatcaggtgcgacaatctatcgattgtatgggaagcccgatgcgccagagttgtttctgaaacatggcaaaggtagcgttgccaatgatgttacagatgagatggtcagactaaactggctgacggaatttatgcctcttccgaccatcaagcattttatccgtactcctgatgatgcatggttactcaccactgcgatccccgggaaaacagcattccaggtattagaagaatatcctgattcaggtgaaaatattgttgatgcgctggcagtgttcctgcgccggttgcattcgattcctgtttgtaattgtccttttaacagcgatcgcgtatttcgtctcgctcaggcgcaatcacgaatgaataacggtttggttgatgcgagtgattttgatgacgagcgtaatggctggcctgttgaacaagtctggaaagaaatgcataaacttttgccattctcaccggattcagtcgtcactcatggtgatttctcacttgataaccttatttttgacgaggggaaattaataggttgtattgatgttggacgagtcggaatcgcagaccgataccaggatcttgccatcctatggaactgcctcggtgagttttctccttcattacagaaacggctttttcaaaaatatggtattgataatcctgatatgaataaattgcagtttcatttgatgctcgatgagtttttctaa

SEQ ID NO: 13 - DNA, 105 bp, Artificial Sequence
  AmpR promoter
cgcggaacccctatttgtttatttttctaaatacattcaaatatgtatccgctcatgagacaataaccctgataaatgcttcaataatattgaaaaaggaagagt

SEQ ID NO: 14 - DNA, 87 bp, Artificial Sequence
  rrnB T1 terminator
caaataaaacgaaaggctcagtcgaaagactgggcctttcgttttatctgttgtttgtcggtgaacgctctcctgagtaggacaaat

SEQ ID NO: 15 - DNA, 28 bp, Artificial Sequence
  rrnB T2 terminator
agaaggccatcctgacggatggcctttt

SEQ ID NO: 16 - DNA, 589 bp, Artificial Sequence
  pMB1 origin of replication
tttccataggctccgcccccctgacgagcatcacaaaaatcgacgctcaagtcagaggtggcgaaacccgacaggactataaagataccaggcgtttccccctggaagctccctcgtgcgctctcctgttccgaccctgccgcttaccggatacctgtccgcctttctcccttcgggaagcgtggcgctttctcatagctcacgctgtaggtatctcagttcggtgtaggtcgttcgctccaagctgggctgtgtgcacgaaccccccgttcagcccgaccgctgcgccttatccggtaactatcgtcttgagtccaacccggtaagacacgacttatcgccactggcagcagccactggtaacaggattagcagagcgaggtatgtaggcggtgctacagagttcttgaagtggtggcctaactacggctacactagaaggacagtatttggtatctgcgctctgctgaagccagttaccttcggaaaaagagttggtagctcttgatccggcaaacaaaccaccgctggtagcggtggtttttttgtttgcaagcagcagattacgcgcagaaaaaaaggatctcaa

SEQ ID NO: 17 - DNA, 6088 bp, Artificial Sequence
  KTXHIS-pelbLC-pelbHC
atctttctgcgaattgagatgacgccactggctgggcgtcatcccggtttcccgggtaaacaccaccgaaaaatagttactatcttcaaagccacattcggtcgaaatatcactgattaacaggcggctatgctggagaagatattgcgcatgacacactctgacctgtcgcagatattgattgatggtcattccagtctgctggcgaaattgctgacgcaaaacgcgctcactgcacgatgcctcatcacaaaatttatccagcgcaaagggacttttcaggctagccgccagccgggtaatcagcttatccagcaacgtttcgctggatgttggcggcaacgaatcactggtgtaacgatggcgattcagcaacatcaccaactgcccgaacagcaactcagccatttcgttagcaaacggcacatgctgactactttcatgctcaagctgaccaataacctgccgcgcctgcgccatccccatgctacctaagcgccagtgtggttgccctgcgctggcgttaaatcccggaatcgccccctgccagtcaagattcagcttcagacgctccgggcaataaataatattctgcaaaaccagatcgttaacggaagcgtaggagtgtttatcatcagcatgaatgtaaaagagatcgccacgggtaatgcgataagggcgatcgttgagtacatgcaggccattaccgcgccagacaatcaccagctcacaaaaatcatgtgtatgttcagcaaagacatcttgcggataacggtcagccacagcgactgcctgctggtcgctggcaaaaaaatcatctttgagaagttttaactgatgcgccaccgtggctacctcggccagagaacgaagttgattattcgcaatatggcgtacaaatacgttgagaagattcgcgttattgcagaaagccatcccgtccctggcgaatatcacgcggtgaccagttaaactctcggcgaaaaagcgtcgaaaagtggttactgtcgctgaatccacagcgataggcgatgtcagtaacgctggcctcgctgtggcgtagcagatgtcgggctttcatcagtcgcaggcggttcaggtatcgctgaggcgtcagtcccgtttgctgcttaagctgccgatgtagcgtacgcagtgaaagagaaaattgatccgccacggcatcccaattcacctcatcggcaaaatggtcctccagccaggccagaagcaagttgagacgtgatgcgctgttttccaggttctcctgcaaactgcttttacgcagcaagagcagtaattgcataaacaagatctcgcgactggcggtcgagggtaaatcattttccccttcctgctgttccatctgtgcaaccagctgtcgcacctgctgcaatacgctgtggttaacgcgccagtgagacggatactgcccatccagctcttgtggcagcaactgattcagcccggcgagaaactgaaatcgatccggcgagcgatacagcacattggtcagacacagattatcggtatgttcatacagatgccgatcatgatcgcgtacgaaacagaccgtgccaccggtgatggtatagggctgcccattaaacacatgaatacccgtgccatgttcgacaatcacaatttcatgaaaatcatgatgatgttcaggaaaatccgcctgcgggagccggggttctatcgccacggacgcgttaccagacggaaaaaaatccacactatgtaatacggtcatactggcctcctgatgtcgtcaacacggcgaaatagtaatcacgaggtcaggttcttaccttaaattttcgacggaaaaccacgtaaaaaacgtcgatttttcaagatacagcgtgaattttcaggaaatgcggtgagcatcacatcaccacaattcagcaaattgtgaacatcatcacgttcatctttccctggttgccaatggcccattttcttgtcagtaacgagaaggtcgcgaatccaggcgctttttagactggtcgtaatgaaattcaggaggaattcctaatgaaatatctgctgccgaccgcagcagcgggtctgctgctgctggcagcacagcctgcaatggcagatattcagctgacccagagcccgagcagcctgagcgcaagcgttggtgatcgtgttaccattacctgtagcgcaagccaggatattagcaattatctgaattggtatcagcagaaaccgggtaaagcaccgaaagtgctgatctattttaccagcagcctgcatagcggtgttccgagccgttttagcggtagcggtagtggcaccgattttaccctgaccattagcagcctgcagccggaagattttgcaacctattattgtcagcagtatagcaccgttccgtggacctttggtcagggcaccaaagttgaaattaaacgtaccgttgcagcaccgagcgtttttatctttccgcctagtgatgaacagctgaaaagcggcaccgcaagcgttgtttgtctgctgaataacttttatccgcgtgaagcaaaagttcagtggaaagttgataatgcactgcagagcggtaatagccaagaaagcgttaccgaacaggatagcaaagatagcacctatagcctgagcagcaccctgaccctgagcaaagcagattatgaaaaacacaaagtgtatgcctgcgaagttacccatcagggtctgagcagtccggttaccaaaagttttaatcgtggtgaatgctaataatctagaactgttatcgatatcaggaggattagcatatgaaatatctgctgccgaccgcagcagcgggtctgctgctgctggcagcacagcctgcaatggcagaagttcagctggttgaaagcggtggtggtctggttcagcctggtggtagcctgcgtctgagctgtgcagcaagcggttatgattttacccattatggtatgaattgggttcgtcaggcaccgggtaaaggtctggaatgggttggttggattaatacctataccggtgaaccgacctatgcagcagattttaaacgtcgttttacctttagcctggataccagcaaaagcaccgcatatctgcagatgaatagcctgcgtgcagaggataccgcagtgtattattgtgcaaaatatccgtattattacggcaccagccattggtatttcgatgtttggggtcagggcaccctggttaccgttagcagcgcaagcaccaaaggtccgagcgtttttccgctggcaccgagcagcaaaagtaccagcggtggcaccgcagcactgggttgtctggttaaagattattttccggaaccggttaccgtgagctggaatagcggtgcactgaccagcggtgttcatacctttccggcagttctgcagagcagcggtctgtatagcctgagcagcgttgttaccgttccgagcagcagcctgggcacccagacctatatttgtaatgttaatcataaaccgagcaataccaaagtggataaaaaagtggaaccgaaaagctgcgataaaacccatctgtaataaaagcttggctgttttggcggatgagagaagattttcagcctgatacagattaaatcagaacgcagaagcggtctgataaaacagaatttgcctggcggcagtagcgcggtggtcccacctgaccccatgccgaactcagaagtgaaacgccgtagcgccgatggtagtgtggggtctccccatgcgagagtagggaactgccaggcatcaaataaaacgaaaggctcagtcgaaagactgggcctttcgttttatctgttgtttgtcggtgaacgctctcctgagtaggacaaatccgccgggagcggatttgaacgttgcgaagcaacggcccggagggtggcgggcaggacgcccgccataaactgccaggcatcaaattaagcagaaggccatcctgacggatggcctttttgcgtttctacaaactcttttgtttatttttctaaatacattcaaatatgtatccgctcatgagactaggcttccgcgccctcatccgaaagggcgtattcatatatgcggtgtgaaataccgcacagatgcgtaaggagaaaataccgcatcaggcgctcttccgcttcctcgctcactgactcgctgcgctcggtcgttcggctgcggcgagcggtatcagctcactcaaaggcggtaatacggttatccacagaatcaggggataacgcaggaaagaacatgtgagcaaaaggccagcaaaaggccaggaaccgtaaaaaggccgcgttgctggcgtttttccataggctccgcccccctgacgagcatcacaaaaatcgacgctcaagtcagaggtggcgaaacccgacaggactataaagataccaggcgtttccccctggaagctccctcgtgcgctctcctgttccgaccctgccgcttaccggatacctgtccgcctttctcccttcgggaagcgtggcgctttctcatagctcacgctgtaggtatctcagttcggtgtaggtcgttcgctccaagctgggctgtgtgcacgaaccccccgttcagcccgaccgctgcgccttatccggtaactatcgtcttgagtccaacccggtaagacacgacttatcgccactggcagcagccactggtaacaggattagcagagcgaggtatgtaggcggtgctacagagttcttgaagtggtggcctaactacggctacactagaaggacagtatttggtatctgcgctctgctgaagccagttaccttcggaaaaagagttggtagctcttgatccggcaaacaaaccaccgctggtagcggtggtttttttgtttgcaagcagcagattacgcgcagaaaaaaaggatctcaagaagatcctttgatcttttctacggggtctgacgctcagtggaacgaaaactcacgttaagggattttggtcatgagattatcaaaaaggatcttcacctagatccttttaaattaaaaatgaagttttaaatcaatctaaagtatatatgagtaaacttggtctgacagttagaaaaactcatcgagcatcaaatgaaactgcaatttattcatatcaggattatcaataccatatttttgaaaaagccgtttctgtaatgaaggagaaaactcaccgaggcagttccataggatggcaagatcctggtatcggtctgcgattccgactcgtccaacatcaatacaacctattaatttcccctcgtcaaaaataaggttatcaagtgagaaatcaccatgagtgacgactgaatccggtgagaatggcaaaagtttatgcatttctttccagacttgttcaacaggccagccattacgctcgtcatcaaaatcactcgcatcaaccaaaccgttattcattcgtgattgcgcctgagcgagacgaaatacgcgatcgctgttaaaaggacaattacaaacaggaatcgaatgcaaccggcgcaggaacactgccagcgcatcaacaatattttcacctgaatcaggatattcttctaatacctggaatgctgttttcccggggatcgcagtggtgagtaaccatgcatcatcaggagtacggataaaatgcttgatggtcggaagaggcataaattccgtcagccagtttagtctgaccatctcatctgtaacatcattggcaacgctacctttgccatgtttcagaaacaactctggcgcatcgggcttcccatacaatcgatagattgtcgcacctgattgcccgacattatcgcgagcccatttatacccatataaatcagcatccatgttggaatttaatcgcggcctagagcaagacgtttcccgttgaatatggctcatactcttcctttttcaatattattgaagcatttatcagggttattgtctcatgagcggatacatatttgaatgtatttagaaaaataaacaaataggggttccgcgcacatttccccgaaaagtgccacctgacgtctaagaaaccattattatcatgacattaacctataaaaataggcgtatcacgaggccctttcgtct

SEQ ID NO: 18 - protein, 22 aa, Erwinia
  PelB signal peptide - peptide
MKYLLPTAAAGLLLLAAQPAMA

SEQ ID NO: 19 - DNA, 32 bp, Artificial Sequence
  SBamHI1680
gtacgctaggatcctgtggcagcaactgattc

SEQ ID NO: 20 - DNA, 32 bp, Artificial Sequence
  BSalI1681
gtagataggtcgacagcgatcgtcattgggat

SEQ ID NO: 21 - DNA, 180 bp, Artificial Sequence
  Figure 2 - Multiple cloning site
gagaaggtcgcgaatccaggcgctttttagactggtcgtaatgaaattcaggaggaattccatatggcggccgcactcgagcaccaccaccaccaccactgatgaagacggccgcctaggggtaccgagctcggatcctctagagtcgacctgcaggcatgcaagcttggctgttttggc